European Patent Application EP 4 372 378 A1, published May 22, 2024. Title: METHOD FOR DETECTING HEPATITIS E VIRUS INFECTION, AND ANTIGEN POLYPEPTIDE AND KIT FOR DETECTING HEPATITIS E VIRUS INFECTION. Applicant: Advanced Life Science Institute Inc. Application JP. The sequence listing filed with the application follows.

SEQUENCE LISTING (20 sequences)

SEQ ID NO: 1 - protein, 229 aa, Hepatitis E virus
DLGESRVVIQDYDNQHEQDRPTPSPAPSRPFSVLRANDVLWLSLTAAEYDQSTYGSSTGPVYVSDSVTLVNVATGAQAVARSLDWTKVTLDGRPLSTIQQYSKTFFVLPLRGKLSFWEAGTTKAGYPYNYNTTASDQLLVENAAGHRVAISTYTTSLGAGPVSISAVAVLAPHSALALLEDTMDYPARAHTFDDFCPECRPLGLQGCAFQSTVAELQRLKMKVGKTREL

SEQ ID NO: 2 - protein, 229 aa, Hepatitis E virus
DLGDSRVVIQDYDNQHEQDRPTPSPAPSRPFSVLRANDVLWLSLTAAEYDQSTYGSSTGPVYISDSVTLVNVATGAQAVARSLDWSKVTLDGRPLPTVEQYSKTFFVLPLRGKLSFWEAGTTKAGYPYNYNTTASDQILIENAAGHRVAISTYTTRLGAGPVAISAAAVLAPRSALALLEDTFDYPGRAHTFDDFCPECRALGLQGCAFQSTVAELQRLKVKVGKTREL

SEQ ID NO: 3 - protein, 229 aa, Hepatitis E virus
DLGDSRVVIQDYDNQHEQDRPTPSPAPSRPFSVLRANDVLWLSLTAAEYDQTTYGSSTNPMYVSDTVTFVNVATGAQAVARSLDWSKVTLDGRPLTTIQQYSKTFYVLPLRGKLSFWEAGTTKAGYPYNYNTTASDQILIENAAGHRVAISTYTTSLGAGPTSISAVGVLAPHSALAVLEDTADYPARAHTFDDFCPECRALGLQGCAFQSTIAELQRLKTKVGKTREF

SEQ ID NO: 4 - protein, 229 aa, Hepatitis E virus
DLGESRVVIQDYDNQHEQDRPTPSPAPSRPFSVLRANDVLWLSLTAAEYDQTTYGSSTNPMYVSDTVTFVNVATGAQGVSRSLDWSKVTFDGRPLTTIQQYSKTFFVLPLRGKLSFWEAGTTKAGYPYNYNTTASDQILIENAAGHRVCISTYTTNLGSGPVSISAVGVLAPHSALAALEDTVDYPARAHTFDDFCPECRTLGLQGCAFQSTVAELQRLKMKVGKTREY

SEQ ID NO: 5 - DNA, 27 bp, synthetic construct
  misc_feature 1..27: note = reverse primer G3AS1
  source 1..27: mol_type = other DNA
gtacaaaaagaattaattaaaactccc

SEQ ID NO: 6 - DNA, 30 bp, synthetic construct
  misc_feature 1..30: note = primer G3S1
  source 1..30: mol_type = other DNA
atcatacagcgggtggaatgaataacatgt

SEQ ID NO: 7 - DNA, 25 bp, synthetic construct
  misc_feature 1..25: note = primer G3S2
  source 1..25: mol_type = other DNA
acagcgggtggaatgaataacatgt

SEQ ID NO: 8 - DNA, 29 bp, synthetic construct
  misc_feature 1..29: note = primer G3AS2
  source 1..29: mol_type = other DNA
aattaattaaaactcccgggttttaccta

SEQ ID NO: 9 - DNA, 49 bp, synthetic construct
  misc_feature 1..49: note = primer G3E2s-his452-S
  source 1..49: mol_type = other DNA
tatgaattccatcatcatcatcatcatcctactccttcacccgccccct

SEQ ID NO: 10 - DNA, 42 bp, synthetic construct
  misc_feature 1..42: note = primer G3E2s-617-AS
  source 1..42: mol_type = other DNA
atgggatccttagggatagtcagcagtgtcctcaagaacggc

SEQ ID NO: 11 - DNA, 31 bp, synthetic construct
  misc_feature 1..31: note = primer G3E2s-452-S
  source 1..31: mol_type = other DNA
tatgaattccctactccttcacccgccccct

SEQ ID NO: 12 - DNA, 687 bp, synthetic construct
  misc_feature 1..687: note = G1E2s 394-617
  source 1..687: mol_type = other DNA
gaattccaactgttctatagccgtccagttgtgagcgccaatggagaaccgacggtcaagctgtacacctccgttgagaatgcccaacaggacaaaggcattgcgattcctcacgacatcgacttaggggaatcacgggtggtgatccaggattacgacaaccagcacgaacaagatcgccctaccccgagtccagcgccgtcacgcccctttagtgtgctccgtgccaacgatgtactctggctgagcctgacagcagcggaatacgatcagagtacctatggctccagcactggtccggtgtatgtgagcgattcagtaaccctggtcaatgtcgcaacaggagctcaagcagtagcgcgtagcttggattggacgaaagtcaccctggatggtcgcccgttatcgacgatccagcagtactcgaaaaccttctttgtgcttccattgcgcggcaaactgtcgttttgggaagcggggactacgaaagcgggctatccgtataactacaacacgactgcctctgatcagctgttagtcgagaatgcggcaggccatcgcgttgcgatttccacctataccacatctctgggtgctggtcccgtgtcgattagtgccgttgctgttcttgcaccgcattctgccctggctttgctggaagataccatggactatccgtaaggatcc

SEQ ID NO: 13 - DNA, 48 bp, synthetic construct
  misc_feature 1..48: note = primer G1E2s-his452-S
  source 1..48: mol_type = other DNA
gaattccatcatcatcatcatcataccccgagtccagcgccgtcacgc

SEQ ID NO: 14 - DNA, 21 bp, synthetic construct
  misc_feature 1..21: note = primer G1E2s-617-AS
  source 1..21: mol_type = other DNA
ggatccttacggatagtccat

SEQ ID NO: 15 - DNA, 29 bp, synthetic construct
  misc_feature 1..29: note = reverse primer G4AS1
  source 1..29: mol_type = other DNA
ggaaggtacaagcaaaataaatcaatact

SEQ ID NO: 16 - DNA, 27 bp, synthetic construct
  misc_feature 1..27: note = primer G4S1
  source 1..27: mol_type = other DNA
tagctctattatataccgggtggaatg

SEQ ID NO: 17 - DNA, 27 bp, synthetic construct
  misc_feature 1..27: note = primer G4S2
  source 1..27: mol_type = other DNA
ataccgggtggaatgaataacatgttc

SEQ ID NO: 18 - DNA, 28 bp, synthetic construct
  misc_feature 1..28: note = primer G4AS2
  source 1..28: mol_type = other DNA
gtacaagcaaaataaatcaatactcccg

SEQ ID NO: 19 - DNA, 49 bp, synthetic construct
  misc_feature 1..49: note = primer G4E2s-his445-S
  source 1..49: mol_type = other DNA
tgaattccatcatcatcatcatcataaccagcatgagcaggaccgtccc

SEQ ID NO: 20 - DNA, 42 bp, synthetic construct
  misc_feature 1..42: note = primer G4E2s-606-AS
  source 1..42: mol_type = other DNA
taaggatccttatgcagagtgaggtgcaaggacaccgacagc